European Patent Application EP 4 481 386 A1, published December 25, 2024. Title: Implantable apparatuses, biosensor devices, systems and methods. Applicant: IMPLI LIMITED IMPLANTABLE HEALTHCARE. The sequence listing filed with the application follows.

SEQUENCE LISTING (4 sequences)

SEQ ID NO: 1 - DNA, 35 bp, synthetic construct
  source 1..35: mol_type = other DNA
tatggtatgctgtgtggtatggggtggcgtgctct

SEQ ID NO: 2 - DNA, 48 bp, synthetic construct
  source 1..48: mol_type = other DNA
tttttttttttttttgcttccagcttattgaattacacgcagagggta

SEQ ID NO: 3 - DNA, 55 bp, synthetic construct
  source 1..55: mol_type = other DNA
gcggctctgcgcattcaattgctgcgcgctgaagcgcggaagctttttttttttt

SEQ ID NO: 4 - DNA, 60 bp, synthetic construct
  source 1..60: mol_type = other DNA
gcatcacacaccgatactcacccgcctgattaacattagcccaccgcccacccccgctgc